European Patent Specification EP 3 430 039 B1, published October 22, 2025. Title: ENGINEERED IMMUNOGLOBULINS WITH ALTERED FCRN BINDING. Applicant: UNIVERSITY OF OSLO. The sequence listing filed with the application follows.

SEQUENCE LISTING (16 sequences)

SEQ ID NO: 1 - protein, 330 aa, Artificial Sequence [sequence omitted]

SEQ ID NO: 2 - protein, 330 aa, Artificial Sequence
  synthetic
ASTKGPSVFPLAPSSKSTSGGTAALGCLVKDYFPEPVTVSWNSGALTSGVHTFPAVLQSSGLYSLSSVVTVPSSSLGTQTYICNVNHKPSNTKVDKKVEPKSCDKTHTCPPCPAPELLGGPSVFLFPPKPKDTLMISRTPEVTCVVVDVSHEDPEVKFNWYVDGVEVHNAKTKPREEQYNSTYRVVSVLTVLHRDWLNGKEYKCKVSNKALPAPIEKTISKAKGQPREPQVYTLPPSRDELTKNQVSLTCLVKGFYPSDIAVEWESNGQPENNYKTTPPVLDSDGSFFLYSKLTVDKSRWQQGNVFSCSVEHEALHWHYTQKSLSLSPGK

SEQ ID NO: 3 - protein, 330 aa, Artificial Sequence
  synthetic
ASTKGPSVFPLAPSSKSTSGGTAALGCLVKDYFPEPVTVSWNSGALTSGVHTFPAVLQSSGLYSLSSVVTVPSSSLGTQTYICNVNHKPSNTKVDKKVEPKSCDKTHTCPPCPAPELLGGPSVFLFPPKPKDTLMISRTPEVTCVVVDVSHEDPEVKFNWYVDGVEVHNAKTKPREEQYNSTYRVVSVLTVLHRDWLNGKEYKCKVSNKALPAPIEKTISKAKGQPREPQVYTLPPSRDELTKNQVSLTCLVKGFYPSDIAVEWESNGQPENNYKTTPPVLDSDGSFFLYSKLTVDKSRWQQGNVFSCSVMHEALHWHYTQKSLSLSPGK

SEQ ID NO: 4 - protein, 330 aa, Artificial Sequence
  synthetic
ASTKGPSVFPLAPSSKSTSGGTAALGCLVKDYFPEPVTVSWNSGALTSGVHTFPAVLQSSGLYSLSSVVTVPSSSLGTQTYICNVNHKPSNTKVDKKVEPKSCDKTHTCPPCPAPELLGGPSVFLFPPKPKDTLMISRTPEVTCVVVDVSHEDPEVKFNWYVDGVEVHNAKTKPREEQYNSTYRVVSVLTVLHRDWLNGKEYKCKVSNKALPAPIEKTISKAKGQPREPQVYTLPPSRDELTKNQVSLTCLVKGFYPSDIAVEWESNGQPENNYKTTPPVLDSDGSFFLYSKLTVDKSRWQQGNVFSCSVMHEALHNHYTQKSLSLSPGK

SEQ ID NO: 5 - protein, 330 aa, Artificial Sequence
  synthetic
ASTKGPSVFPLAPSSKSTSGGTAALGCLVKDYFPEPVTVSWNSGALTSGVHTFPAVLQSSGLYSLSSVVTVPSSSLGTQTYICNVNHKPSNTKVDKKVEPKSCDKTHTCPPCPAPELLGGPSVFLFPPKPKDTLMISRTPEVTCVVVDVSHEDPEVKFNWYVDGVEVHNAKTKPREEQYNSTYRVVSVLTVLHQDWLNGKEYKCKVSNKALPAPIEKTISKAKGQPREPQVYTLPPSRDELTKNQVSLTCLVKGFYPSDIAVEWESNGQPENNYKTTPPVLDSDGSFFLYSKLTVDKSRWQQGNVFSCSVMHEALHWHYTQKSLSLSPGK

SEQ ID NO: 6 - protein, 330 aa, Artificial Sequence [sequence omitted]

SEQ ID NO: 7 - protein, 330 aa, Artificial Sequence; identical to SEQ ID NO: 2
  synthetic

SEQ ID NO: 8 - protein, 330 aa, Artificial Sequence
  synthetic
ASTKGPSVFPLAPSSKSTSGGTAALGCLVKDYFPEPVTVSWNSGALTSGVHTFPAVLQSSGLYSLSSVVTVPSSSLGTQTYICNVNHKPSNTKVDKKVEPKSCDKTHTCPPCPAPELLGGPSVFLFPPKPKDTLSISRTPEVTCVVVDVSHEDPEVKFNWYVDGVEVHNAKTKPREEQYNSTYRVVSVLTVLHRDWLNGKEYKCKVSNKALPAPIEKTISKAKGQPREPQVYTLPPSRDELTKNQVSLTCLVKGFYPSDIAVEWESNGQPENNYKTTPPVLDSDGSFFLYSKLTVDKSRWQQGNVFSCSVEHEALHWHYTQKSLSLSPGK

SEQ ID NO: 9 - protein, 330 aa, Artificial Sequence
  synthetic
ASTKGPSVFPLAPSSKSTSGGTAALGCLVKDYFPEPVTVSWNSGALTSGVHTFPAVLQSSGLYSLSSVVTVPSSSLGTQTYICNVNHKPSNTKVDKKVEPKSCDKTHTCPPCPAPELLGGPSVFLFPPKPKDTLMISRTPEVTCVVVDVSHEDPEVKFNWYVDGVEVHNAKTKPREEQYNSTYRVVSVLTVLHRDWLNGKEYKCKVSNKALPAPIEKTISKAKGQPREPQVYTLPPSRDELTKNQVSLTCLVKGFYPSDIAVEWESNGQPENNYKTTPPVLDSDGSFFLYSKLTVDKSRWQQGNVFSCSVEHEALHPHYTQKSLSLSPGK

SEQ ID NO: 10 - protein, 330 aa, Artificial Sequence
  synthetic
ASTKGPSVFPLAPSSKSTSGGTAALGCLVKDYFPEPVTVSWNSGALTSGVHTFPAVLQSSGLYSLSSVVTVPSSSLGTQTYICNVNHKPSNTKVDKKVEPKSCDKTHTCPPCPAPELLGGPSVFLFPPKPKDTLMISRTPEVTCVVVDVSHEDPEVKFNWYVDGVEVHNAKTKPREEQYNSTYRVVSVLTVLHRDWLNGKEYKCKVSNKALPAPIEKTISKAKGQPREPQVYTLPPSRDELTKNQVSLTCLVKGFYPSDIAVEWESNGQPENNYKTTPPVLDSDGSFFLYSKLTVDKSRWQQGNVFSCSVDHEALHWHYTQKSLSLSPGK

SEQ ID NO: 11 - protein, 330 aa, Artificial Sequence
  synthetic
ASTKGPSVFPLAPSSKSTSGGTAALGCLVKDYFPEPVTVSWNSGALTSGVHTFPAVLQSSGLYSLSSVVTVPSSSLGTQTYICNVNHKPSNTKVDKKVEPKSCDKTHTCPPCPAPELLGGPSVFLFPPKPKDTLMISRTPEVTCVVVDVSHEDPEVKFNWYVDGVEVHNAKTKPREEQYNSTYRVVSVLTVLHRDWLNGKEYKCKVSNKALPAPIEKTISKAKGQPREPQVYTLPPSRDELTKNQVSLTCLVKGFYPSDIAVEWESNGQPENNYKTTPPVLDSDGSFFLYSKLTVDKSRWQQGNVFSCSVEHEALKWHYTQKSLSLSPGK

SEQ ID NO: 12 - protein, 330 aa, Artificial Sequence
  synthetic
ASTKGPSVFPLAPSSKSTSGGTAALGCLVKDYFPEPVTVSWNSGALTSGVHTFPAVLQSSGLYSLSSVVTVPSSSLGTQTYICNVNHKPSNTKVDKKVEPKSCDKTHTCPPCPAPELLGGPSVFLFPPKPKDTLMISRTPEVTCVVVDVSHEDPEVKFNWYVDGVEVHNAKTKPREEQYNSTYRVVSVLTVKHRDWLNGKEYKCKVSNKALPAPIEKTISKAKGQPREPQVYTLPPSRDELTKNQVSLTCLVKGFYPSDIAVEWESNGQPENNYKTTPPVLDSDGSFFLYSKLTVDKSRWQQGNVFSCSVEHEALHWHYTQKSLSLSPGK

SEQ ID NO: 13 - protein, 330 aa, Artificial Sequence
  synthetic
ASTKGPSVFPLAPSSKSTSGGTAALGCLVKDYFPEPVTVSWNSGALTSGVHTFPAVLQSSGLYSLSSVVTVPSSSLGTQTYICNVNHKPSNTKVDKKVEPKSCDKTHTCPPCPAPELLGGPSVFLFPPKPKDTLMISRTPEVTCVVVDVSHEDPEVKFNWYVDGVEVHNAKTKPREEQYNSTYRVVSVLTVRHRDWLNGKEYKCKVSNKALPAPIEKTISKAKGQPREPQVYTLPPSRDELTKNQVSLTCLVKGFYPSDIAVEWESNGQPENNYKTTPPVLDSDGSFFLYSKLTVDKSRWQQGNVFSCSVEHEALHWHYTQKSLSLSPGK

SEQ ID NO: 14 - protein, 330 aa, Artificial Sequence
  synthetic
ASTKGPSVFPLAPSSKSTSGGTAALGCLVKDYFPEPVTVSWNSGALTSGVHTFPAVLQSSGLYSLSSVVTVPSSSLGTQTYICNVNHKPSNTKVDKKVEPKSCDKTHTCPPCPAPELLGGPSVFLFPPKPKDTLMISRTPEVTCVVVDVSHEDPEVKFNWYVDGVEVHNAKTKPREEQYNSTYRVVSVLTVSHRDWLNGKEYKCKVSNKALPAPIEKTISKAKGQPREPQVYTLPPSRDELTKNQVSLTCLVKGFYPSDIAVEWESNGQPENNYKTTPPVLDSDGSFFLYSKLTVDKSRWQQGNVFSCSVEHEALHWHYTQKSLSLSPGK

SEQ ID NO: 15 - protein, 377 aa, Artificial Sequence
  synthetic
ASTKGPSVFPLAPCSRSTSGGTAALGCLVKDYFPEPVTVSWNSGALTSGVHTFPAVLQSSGLYSLSSVVTVPSSSLGTQTYTCNVNHKPSNTKVDKRVELKTPLGDTTHTCPRCPEPKSCDTPPPCPRCPEPKSCDTPPPCPRCPEPKSCDTPPPCPRCPAPELLGGPSVFLFPPKPKDTLMISRTPEVTCVVVDVSHEDPEVQFKWYVDGVEVHNAKTKPREEQYNSTFRVVSVLTVLHRDWLNGKEYKCKVSNKALPAPIEKTISKTKGQPREPQVYTLPPSREEMTKNQVSLTCLVKGFYPSDIAVEWESSGQPENNYNTTPPMLDSDGSFFLYSKLTVDKSRWQQGNIFSCSVEHEALHWHFTQKSLSLSPGK

SEQ ID NO: 16 - protein, 377 aa, Artificial Sequence; identical to SEQ ID NO: 15
  synthetic